European Patent Application EP 4 360 629 A1, published May 1, 2024. Title: Pharmaceutical composition containing lipolytic enzyme inhibitors for preventing or treating RNA virus infection. Applicant: INDUSTRY FOUNDATION OF CHONNAM NATIONAL UNIVERSITY. The sequence listing filed with the application follows.

SEQUENCE LISTING (22 sequences)

SEQ ID NO: 1 - DNA, 22 bp, Artificial Sequence
  SARS-CoV-2 N F
taatcagacaaggaactgatta

SEQ ID NO: 2 - DNA, 19 bp, Artificial Sequence
  SARS-CoV-2 N R
cgaaggtgtgacttccatg

SEQ ID NO: 3 - DNA, 20 bp, Artificial Sequence
  IAV PB1 F
ctgccagaagacaatgaacc

SEQ ID NO: 4 - DNA, 20 bp, Artificial Sequence
  IAV PB1 R
ggccattgcttccaatacac

SEQ ID NO: 5 - DNA, 24 bp, Artificial Sequence
  RVA VP6 F
tagaccaaataacgttgaagttga

SEQ ID NO: 6 - DNA, 22 bp, Artificial Sequence
  RVA VP6 R
gattcacaaactgcagattcaa

SEQ ID NO: 7 - DNA, 20 bp, Artificial Sequence
  PEDV F
gctatgctcagatcgccagt

SEQ ID NO: 8 - DNA, 22 bp, Artificial Sequence
  PEDV R
tctcgtaagagtccgctagctc

SEQ ID NO: 9 - DNA, 19 bp, Artificial Sequence
  PRRSV M F
cacctccagatgccgtttg

SEQ ID NO: 10 - DNA, 20 bp, Artificial Sequence
  PRRSV M R
atgcgtggttatcatttgcc

SEQ ID NO: 11 - DNA, 20 bp, Artificial Sequence
  PSaV VPg F
cgaaagggaaaaacaaacgc

SEQ ID NO: 12 - DNA, 24 bp, Artificial Sequence
  PSaV VPg R
tcactcactgtcataggtgtcacc

SEQ ID NO: 13 - DNA, 21 bp, Artificial Sequence
  BCoV N F
tggatcaagattagagttggc

SEQ ID NO: 14 - DNA, 20 bp, Artificial Sequence
  BCoV N R
ccttgtccattcttctgacc

SEQ ID NO: 15 - DNA, 20 bp, Artificial Sequence
  L32 F
tctggtgaagcccaagatcg

SEQ ID NO: 16 - DNA, 18 bp, Artificial Sequence
  L32 R
ctctgggtttccgccagt

SEQ ID NO: 17 - DNA, 20 bp, Artificial Sequence
  Human GAPDH F
attccacccatggcaaattc

SEQ ID NO: 18 - DNA, 20 bp, Artificial Sequence
  Human GAPDH R
cgctcctggaagatggtgat

SEQ ID NO: 19 - DNA, 20 bp, Artificial Sequence
  Mouse GAPDH F
aaggtcatcccagagctgaa

SEQ ID NO: 20 - DNA, 20 bp, Artificial Sequence
  Mouse GAPDH R
ctgcttcaccaccttcttga

SEQ ID NO: 21 - DNA, 21 bp, Artificial Sequence
  Porcine GAPDH F
acctccactacatggtctaca

SEQ ID NO: 22 - DNA, 20 bp, Artificial Sequence
  Porcine GAPDH R
atgacaagcttcccgttctc